European Patent Specification EP 3 870 195 B9, published October 4, 2023. Title: New probiotics useful for eradicating helicobacter pylori infection. Applicant: VAIRA Berardino. The sequence listing filed with the application follows.

SEQUENCE LISTING (1 sequence)

SEQ ID NO: 1 - DNA, 13 bp, Lactobacillus acidophilus
gtcacgtagttgt